European Patent Application EP 4 279 613 A2, published November 22, 2023. Title: COMPOSITIONS AND METHODS FOR DETECTING OR QUANTIFYING PARAINFLUENZA VIRUS. Applicant: Gen-Probe Incorporated. Application EP. The sequence listing filed with the application follows.

SEQUENCE LISTING (125 sequences)

SEQ ID NO: 1 - DNA, 1000 bp, Human parainfluenza virus 1
  source 1..1000: mol_type = other DNA
tgaagacaaacaccatgacagtatcctccgtgaacgaaagtgccaaaacaatcaaagagacaatcacagaattaatcagacaagaagtgatatcaaggactataaacatacaaagttcagtacaaagcgggatcccaatattgttaaacaagcaaagcagagatctcacacaattaatagagaagtcatgcaacaaacaggaattggctcagatatgcgagaacactattgctattcaccatgcagacggaataacccctctggacccacatgatttctggagatgtcccgtaggagaacccctattgagcaacaaccctaatatctcattattacctggaccaagtctactttctggatcttccacaatttcaggatgtgtcagactaccttcattatcaattggtgatgcaatatatgcgtattcatcaaacttaatcactcaaggatgtgcagatatagggaagtcatatcaggttttacaattaggttacatatctttaaattcagatatgtatcctgatttaaacctggtaatttctcatacctatgacatcaatgacaacaggaaatcatgttctgtaatagctgcaggaacaaggggttaccagttatgctccttgcccactgtgaatgagactacagattactcgagtgaaggtatagaagacttagtatttgacatattagatctcaaaggaaagaccaaatctcatcgatacaaaaatgaagatataacttttgaccatcctttttctgcaatgtatccaagtgtaggaagtgggataaagattgaagatacactcgttttcctaggatatggtggcttaacaactccgcttcaaggcaacaccaagtgtgtgataagcaaatgtcccaatgttaatcagagtgtttgcaatgatgctcttaagataacttggctaaagaaaagacaagttgtcaatgtcttaattcgtatcaataattatttatctgataggccaaagattgttgtcga

SEQ ID NO: 2 - DNA, 500 bp, Human parainfluenza virus 2
  source 1..500: mol_type = other DNA
atcattgaggctcaatgggtaccgtcctatcaagttcctcgtcctggagtcatgccatgcaatgcaacaagtttttgccctgctaattgcatcacaggggtgtacgcagatgtgtggccgcttaatgatccagaactcatgtcacgtaatgctctgaaccccaactatcgatttgctggagcctttctcaaaaatgagtccaaccgaactaatcccacattctacactgcatcggctaactccctcttaaatactaccggattcaacaacaccaatcacaaagcagcatatacatcttcaacctgctttaaaaacactggaacccaaaaaatttattgtttaataataattgaaatgggctcatctcttttaggggagttccaaataataccatttttaagggaactaatgctttaatcctattgaatgaagactccagattcaagaataattggaaggctctttattttatgcgatagttatacgttttggctgtatta

SEQ ID NO: 3 - DNA, 500 bp, Human parainfluenza virus 3
  source 1..500: mol_type = other DNA
tcatagtccatggttttcagatagaaggatggtcaattctataattgttgttgacaagggcttaaactcagttccaaaattgaaggtatggacgatatctatgagacaaaattactgggggtcagaaggaagattacttctactaggtaacaagatctacatatacacaagatctacaagttggcacagcaagttacaattaggaataattgacattactgactacagtgacataaggataaaatggacatggcataatgtgctatcaagaccaggaaacaatgaatgtccatggggacattcatgtccggatgggtgtataacaggagtatatactgatgcatatccactcaatcccacaggaagcattgtatcatctgtcatattggactcacaaaaatcgagagtcaacccagtcataacttactcaacagcaaccgaaagggtgaacgagctggccattcggaacaaaacactctcagctgggtatacaacaacaa

SEQ ID NO: 4 - DNA, 11600 bp, Human parainfluenza virus 4
  source 1..11600: mol_type = other DNA
tccagagatttgcctatcagccttgccgataggacagtatttgtatctagagaagcagaacatgcagtgtgtgacgatatggatacatacctgaataggatattcagtgtattaatacagatttggataatggtgtgcaaatgtatgacagcctatgatcaacccactggatctgaagagagaaggttggctaagtacaagcagcagggcaggatgttagagaaatatcaactgcaaacagatgcaaggaaaattatccaattagtaataagagagagtatggttataagacaatttcttgtacaggagatgttaacagctgataaagtaggtgcttatactaatagatattatgctatggtaggagatattgcaaagtatatagccaatgtcggaatgagtgcattctttcttacactcaagttcggtttgggtaacaggtggaaaccacttgctctagctgcattttctggtgagttagttaaactaaagtctcttatgtcattatacagaagattaggtgacagatcaagatatttggctctcttagaatctcctgaattgatggaatttgctccagccaattacccgctattattcagttacgccatgggagttggaagtgtccaggatccattgatcagaaactatcagtttggaaggaacttcttaaacaccagctattttcagtatggtgttgagactgcaatgaaacaccagggtacagttgaccctaaattggccttagagcttggaataactgatgaagacagagtggatattatgcagtccgttgaaaagcacatatcaggaaaagctggtgatgatatatcacagcctgcaggtgcatttgcaatgtctctaaacagatcagctttcattaacaacaacacttcccaagacttctcaggggcaagactctccaactacgagcaaggatggtccggcacaaatcaagatgaaacgagagatgcctatccagaacctacaatgcatagactccaaaacattgaatcaactgactcagatcacaatgaactactgatgccggagcttgaaagcgacagcaaccccttcaatcgtccaagattcacagtcagagcaccactcatcccagaaatctcgcaccagaatccaaataccagaatgagcagagacatcaacacaagggacaacatcagagctgaccgtcaaaataccaatgaggaccgaggcagcaacattccagatgacattcttggagatctagacaattgacacatcaacaacccagccatagctagacaataatcataaaccgggaaaatctcaaagatacacaatcgcacacatacaatgaaagcaatcacttctgttccacatcacaacccagaaatcctgccaaacgcaacatcacgaccaatcaactgatgatacacagtagaatacaagaacacaactgcattgatttaagaaaaaactaagataggcctgaacggttgcattcaggattctcaatcgttcaggccaatacaattatcagcttcaaacgaaaacaacaagatgagctttgaaataagcatggaggagattgacgagctcattgaaactggcaatctcaacatagattatgcacttaaagaattaggtgcaaccagtcaactcccgccaaataaatctccgtctcagaccagcaaaacagaagaaaccaacgatgagacaagaacctcaaaaaacttggcatcaggagaggcaccagcccacgcctcttcaccactgcggtcacacaatgaagagagtgaatcagggaaacagagcccagacggtttctccatgatatccaacagaccccaaacaggtacactgctcatgggatcagacacacaatctccaagtccatcaaagacctatcaaggactcattcttgatgcaaagaagagagcgctaaatgaaccaaggaggaatcaaaaaacaacaaatgaacatggaaacacaaatgacaccaggatatttaagaggggggaatatagccaccaagaaagaggcttgggttacacaggatcagagatcaaaaacgcaatcttcattccaagacatcgaagggaatactcgatttcatgggtcaacggaagaaccacaatatcagagtggtgcaatccatgttgcgcaccagtcaaaccaaccgcctctgtcgaaaagtgtacatgtggaagatgtcccaaagtttgcgaattgtgcatcagagatccttgatgcaatcaaagcattagaggtgaggttagacaggatcgaagggaaagttgacaaaattatgcttactcaaaatacaattcagcaaacaaaaaatgacactcagcaaattaaaggctcacttgcaacaattgagggcctaatcacaacaatgaaaataatggaccctggagtcccatcaaaagtaagtcttagaagcttaaacaaagggccagagcaagttccaataatcgtcactggtactggcgatgtctcaaaatttgttgatcaagacaatacaattacacttgatccgttagcaagacccattttgtctggaaccaagcaaacaactgatgaaaggagagcaggtgttcgtatagatgcacttaaaataacagtatcagaaatgattcgagatctatttggagactgtgataagagcagaaaacttcttgaatcaataaacatggcaaccacagagcaagaaatcaacttgatcaaaactaatgctcttagaagcatcacttaaactatgagatctatgaatcacgaaggtcacagcgacccagattcactcaatacgccaagcgctcaaccccacacccagaagggacaaccgcaccgcatccccaagaatcgacaccagctcagacgacggcaacaccaatcatcacaaaacaaaacacagaacatcagcactgcatacaaaatcaccccccagcacacacaatccatcgaccgacagattccctccataacattacaaagtatttaagaaaaaaaccagaagtaaggggggacccatcatccaatcgactgtggccatggctcccactcaatccaaagtcaaaattcacaatctagctgaagctcacgagaaggtactgagagccttcccaatagaagttgaacagaactcagaagggaagaaactattagtgaaacagatcagaataagaacgctaggacatgcggatcattcaaatgattcaatttgctttctgaatacttacgggtttatcaaggaagcagtcagccagacagaattcatgagagcaggacagagactagaaagcaaaaacactctgactgcttgcatgttaccctttgggcctggtcctaacatagggtccccccaaaagatgctagaatatgcagaagacattaagatcaatgtaagaaagacagcaggctgcaaggaacagattgtgttttctctagataggacacctcaagtgttcaggggatttcaatttccccgggatagatatgcatgtgttccatctgacaaatatataaaatcaccaggaaagttagtcgcaggacccaattattgttacattatcactttcctttcattgacattctgtcccagcagccagaaattcaaagtacctagacccatattgaattttcgatccacacgaatgaggggtatacatctagagattatcatgaaaattacgtgttctgaaaacagtccaatcagaaagacactaataacagatgatcccgaaaatggaccaaaagcatccgtgtggatccacctctgtaatctttacaaaggaagaaatcctataaaagtatatgatgaggcatattttgcagagaaatgcaaacaaatgctgttaagcgtaggtatcagtgatctatgggggcccacaattgcagtacatgcaaatgggaaaatccccaaatctgccagcctttatttcaactcaagaggatgggctttgcatcccatagctgacgcatctcccacaatggcaaaacaactatggtctataggctgtgagatcattgaagtcaatgcaatattacaaggctctgattacagtgctctggtggatcatcccgatgtaatatatcggaaaatcagaattgatccagcaaaaaagcagtatgcacactctaagtggaatccattcaagaaggcaatatccatgcctgatcttgctggcataaatatctaatcatacaaattaatcactgatatagagttaaggaacattttatattcctccccattgtatcaccatcaccatcccgatatataaaaccacactacactatgcaccgtccaacatccagccaaccacaggatcacaaccacactacaccaactcaatcaaggacatccctgcaaacatcaaacaaccaaaccatgactgtaacagacacagcaccacccgaccaagccagaccctcaccatgcacccaagtcacccgacacaaccgcaaactctcgactctaccattcgacacacatcctcgaacagaccacccaaaaacaccgaacaattaatctcctggtcacaacgatcattgtaaattttaagaaaaaatctaacacacaactagagccaaacacagggggggaaaaacgcatccgccgccacacgcacagatccagaacccaaggcaaccaacacccgtcggactccgctccatcttcaaagaaatcaacatgggtgtcaaaggtctacctctagttatgattggattattaatctcaccaattaccaatttggatataactcatctaatgaatctaggaacggtaccaactgcaattagatctctagtttattacacctacagtaaaccatcctatctcaccgtagatttgattcccaatttgaagaatctagacccaaaatgcaattactcaagtttaaattactacaataaaacggtgttaagcttgattcaaccaattgcagacaatatcaatcaccttacaaagccaatcacaagctcagaaattcaaagtcgtttctttggggcagttataggtacagttgctctcggtgtagctactgctgcacaagttacagcagcaatcggtcttgcaaaagctcaggaaaatgcacgacttatactaactctcaaaaaagctgcagaggaaacaaatgatgcagttcgagatctcatagattccaacaaaattgtggcaaggatgatatcagcaattcagaatcagataaacactgtcattcaacctgccatagaccggattgactgtcaaatcaaagacttacaagctgctaatattttaaatttgtacctaacagagatcacaactgttttccacaatcaattgaccaatcctgcattagaatcaattagtattcaggctctcaaaagtcttctaggatctaccttaccagaagtgctgtctaagttagatctaaacaatatctcggcagcttcagtgatggcatctggcttaattaaaggacagataattgcagttgatataccgactatgacattagtgttgatggtccaaataccaagtatctctcctctacgacaagcaaaaataatagatctaacctctataacaattcacacaaataatcaggaagtacaagctgtggtaccagatagagttcttgagattggttcagagatattaggatttgacggttcagtgtgccaaatcacgaaagatacaatcttttgtccctacaatgatgcatatatattacccatccagcagaaaagatgcctacaaggtcaaacaagagattgcgtgttcaccccggttgctggcacctttcctaggagatttctcactacatatggtactatagtagccaattgcagaaatttagtatgttcttgtctacgacctccccaaataatctaccaacctgatgagaatccagttacaatcatagataaagacttatgtacaacattgactctagactccataactatagagatccagaaatccataaatagtacttttcgacgtgaagtagttctagaatctactcaggttagatctttgactcctcttgatttatcgaccgatttaagtcaatataatcaattactcaagagtgctgaggaccacatccaacggtcaaatgattacttaaactcaatcaatcctagtatagtaaataatagcgcaataataatattgattatactctgcatcttattaatactgacagtcacaatctgcataatttggctcaagtatttgaccaaagaagttaggaatgtagcaagaaatcaaagactcaatagagatgctgatcttatttataagattcccagtcaaattccattgcccagataattgcaaccaagaggcacattttgcaaatcttacccagacgctcctagataaatcgcctacaaagaaaaataaactcccaatttatcaaaagaaatccaaaatcaacggagctacagccatcctgcaataacactgcgaccacaatgatactcttcaagaaatgaaggacaaatccagaaacagaaaaaaatagcccaaaacaaattaacagacagagaaagggagaagcaaacccgtctcagcaaaacctcccatcaacagcactcgaccaagaccgaattaacagcacgaacgcagaaacccactaccacaaaaccacagaaattctcccataatcccccaccaacattcaccaacaaatcagaaaatcattcaaccaggcaacctccacatttcaagtttaagaaaaaaactattataggggggaacgcacttctcagctccaaccacacgaggccttgtcttgtaaaacagaatcaatctcacaaagttcaaaacaaaatctgactacaagtggaacctccacaattcaaaattcaaccaacgatctaacaacaactcatcaactagcaaccatcactgaactcaacaatccagaaggacgtcacatcaattcattcgtgaatctccaaaagaaataacccaagtaaatttacaatctactctttaattataaataaactaaagtaagtcacaaggatgcaagattcacgtggcaatactcaaatattcagccaagcaaattcaatggtaaaaagaacatggagattactattccggattgtaactttaatattacttatttcaatatttgtgttgtcactcataattgtactacaatcaactccagggaatttgcaaagtgatgtcgatataatcagaaaagagctcgatgaacttatggagaactttgaaaccacctctaaatcactgctaagcgtagcaaatcaaattacttatgatgtatcagttctcacccccataaggcaagaagccactgaaacaaacattattgcgaaaataaaagatcattgcaaagatagggtagttaaaggagagagcacctgcacactgggtcacaagcctctacatgatgtttcctttctgaatggatttaacaaattctatttcacatatagggacaatgtacaaatcagacttaatccattattagattatcccaattttattccaactgctacaactcctcatggatgcattcgaattccatcattctccctaagtcaaactcattggtgttatactcacaatacgatcttacggggatgtgaagatacagcatctagcaaacagtatgtatctctaggaaccttacagaccttagaaaatggtgatccttatttcaaggtcgagtacagtcattatttaaatgatagaaagaatcgaaaaagttgctcagtggttgctgtccttgacggatgtttattgtattgtgtgatcatgaccaaaaatgaaacagagaatttcaaggatcctcaattggcaacacaattacttacatatatatcatacaatggtactatcaaagagcgtataataaatccacccggatcatctagagattgggttcacatctcaccaggggtaggttctggtattttgtattcaaattacatcatatttcccttatatggaggccttatggaaaattcaatgatatataataatcaatcagggaaatattttttccctaattcaaccaagttgccatgtagtaataaaaccagtgaaaaaataacaggagcaaaagactcatacacaataacttacttctctaagagacttatacagagtgcatttttgatttgtgatttaagacaatttctttctgaagattgtgaaattttaattcctagcaatgatcacatgctagttggtgcagagggtcgcctatataatattgaaaataatatattttactatcagagaggatccagctggtggccctatccaagcctttatagaatcaaattaaattctaataagaaatatcctagaataattgagatcaaatttacaaaaattgaaatagctccaagacctggcaataaagattgcccaggaaataaagcttgcccaaaagaatgcataacaggagtttaccaagatatatggccactaagttatcctaatactgcgttcccccacaaaaaacgagcgtactatacaggtttttatctcaataattcgcttgcgagacgtaacccgacattttatactgctgacaatctagattaccatcaacaggaaagattgggtaaatttaatcttactgctggatattccactacaacttgtttcaagcagactaccactgcaagattatactgcctttacatacttgaggtgggtgactcagtaattggtgattttcagatttttccctttttacgctcaatagatcaggctatcacttaatcaataggattactctgtaacacaagctgattttataaggtgaaatatgctcatataaaatggtcaatggataaacaataataataatcattataacaaaattaaaaggacaaaacaattacaagaacactatgaactaatcaggaaacaaacatagcattaactaacaacagccaacatgaccaatgacactccatgaaacatcatccatcaataacaaaaagtataatctatcaattagaaccaaacttgatctattctaagtaatctaccaagcgaaaacacacaccaagaatcaccagccatcaaatctgattaatccgacacaaaaatccaaacaaccaccggaacaggcccggtcctgataaacaacctgcccggccaccagcccactcaaaatcaggacacaatcaatttcaccccaatcatcagtttaatccgcaagtcaaacaagtccttccacatgcccagagattcaatcgatctgacacattgctatattttttaagaaaaaagaaaaatgagtgggtgagacattctagttctcatacacagaataaacttcgaaccttggatgcagtatggatcaaaattgaagattgaagaactaggatgattccgcacactaacagacaagcaatgaggaataaaaagaatagacaattgcccaagaggaatgacacaaagcatccaacactaggggggaagagaccacctccaagatggctgatcatactgatgtcctattgccagaggtgcatctgagttcccccattgtacgtcacaaactcatttattatatactattaggaaatttaccaaatcaaataagtcctgaagatcttggacctttatctacaattaattggagccaagttagaagagaagaaagcaaattatgtttacgtttagtatctgtaaggaataatcttttaaaacatataccctcattgagagagatagatccaacacgtcagtgtaaaaatttgtattggccacgacctcttcagttttttaaggatttggatttcaaccaatttaaagggaaaattgaaagatgggaaaaaattcaacacgctacacagcttgtagttaataagagaattatgaattttttagatttaattagtgataaattaatatcaaggaaagacttatttacaagtgctaggtgcagacacgaaggtcatgatagagattcaagattaagagaactagttgatattgaatcgaactggaacaagaatcattggtcaaacactacaaatcttttcttattaataaaatatcaaatgagactgttaatttgtcaaatgaaaaaatctcaaactggtcttcttgaggtcaagttggaagatagatcaggtttaattataattactcccgaattagtgtgtatttatttctataaagcaaatgtattaagctatttcacatttgaaatgatcctcatgatttctgatgtatttgaaggaagacaaaatgtcataggattatgttcagtcagttattacttatctcctctaaaggatagaattaatgacttgcttaattatgtagataatttagcactgattctaggaaataaggtttattcaataatcgctaatttagaaagcttagtttatgctaaattacaattgaaggatccagttttagaagttagaggtcaattccattgttttatactagaagagattatggagatcttacatgatgttttctcagttgatgagagtgctcaagtgtgttctatactgtcatcttttcttagtggtctgtctcctgaccttactgcagaattgttatgtattatgagaatgtggggtcatcccactttaacagctgcaggtgcagcggggaaagtacgtgaatctatgtgtgcaccaaagctactagactttacaacaattatgaaaacattatcattctttcacaccatacttataaatgggtacagaagaaagcatggtgggatctggccaactgtgacgttaattgatggtaccccaaattttattgtcagtctaaaaaatgataatgcagaaataatttatgaagtggcattgaaatactggaaatggatatcactgattgaatttgaaaaatgtttttcagccgatccaggtgaggatttaagtatattcatgaaggataaagcaataagttgtaataagaaggattggatgagtgtattcagacgaagtctcatacatgagagatgtgcaaagaataatttagaatgtccatcaaatgtaaatagaagattgttattaaatttcttaaatgactcaaatttcgatccaaatttagaattagagtatgtaactaccctccagtatctaactgatgataaattttgtgcttcatactctttgaaagaaaaggagataaaagaaactgggagaatatttgcaaagcttacgaagcaaatgagatcgtgtcaagtgataacagaatcaatgcttgctaatcatgcagggaaattattcagagaaaacggtgtagttcttgatcagcttaagttaacaaaatcactcctaactatgagccaaattgggatcatttcaaacaaggagcgtaaagctacaaaggactctatgacaatcctaaaagacattaagaagaataaaaacatacataaagaaaatgaaaagaaatatggttcagagaattcaacccctttcggagactttgggaaaaattttggaataaatactcctgatgattcattagaaatagctgcatgttttttaacaacagatttacaaaagtattgtcttaattggagataccaagcaataataccctttgctagaacattaaatcgaatgtacggatatcctcatct

SEQ ID NO: 5 - DNA, 30 bp, synthetic construct
  misc_feature 1..30: note = Synthetic oligomer
  source 1..30: mol_type = other DNA
ctyacacaattaatagagaagtcatgcaac

SEQ ID NO: 6 - DNA, 23 bp, synthetic construct
  misc_feature 1..23: note = Synthetic oligomer
  source 1..23: mol_type = other DNA
gcaatgtatccaagtgtaggaag

SEQ ID NO: 7 - DNA, 30 bp, synthetic construct
  misc_feature 1..30: note = Synthetic oligomer
  misc_feature 3: note = n is u
  source 1..30: mol_type = other DNA
ctnacacaattaatagagaagtcatgcaac

SEQ ID NO: 8 - DNA, 37 bp, synthetic construct
  misc_feature 1..37: note = Synthetic oligomer
  source 1..37: mol_type = other DNA
cagagatctcacacaattaatagagaagtcatgcaac

SEQ ID NO: 9 - DNA, 37 bp, synthetic construct
  misc_feature 1..37: note = Synthetic oligomer
  source 1..37: mol_type = other DNA
cagagatcttacacaattaatagagaagtcatgcaac

SEQ ID NO: 10 - DNA, 27 bp, synthetic construct
  misc_feature 1..27: note = Synthetic oligomer
  source 1..27: mol_type = other DNA
tacggtggcttaacaactccgctccaa

SEQ ID NO: 11 - DNA, 27 bp, synthetic construct
  misc_feature 1..27: note = Synthetic oligomer
  source 1..27: mol_type = other DNA
tacggtggcttaacaactccgctccaa

SEQ ID NO: 12 - DNA, 30 bp, synthetic construct; identical to SEQ ID NO: 5
  misc_feature 1..30: note = Synthetic oligomer
  source 1..30: mol_type = other DNA

SEQ ID NO: 13 - DNA, 30 bp, synthetic construct; identical to SEQ ID NO: 5
  misc_feature 1..30: note = Synthetic oligomer
  source 1..30: mol_type = other DNA

SEQ ID NO: 14 - DNA, 30 bp, synthetic construct; identical to SEQ ID NO: 7
  misc_feature 1..30: note = Synthetic oligomer
  misc_feature 3: note = n is u
  source 1..30: mol_type = other DNA

SEQ ID NO: 15 - DNA, 30 bp, synthetic construct; identical to SEQ ID NO: 7
  misc_feature 1..30: note = Synthetic oligomer
  misc_feature 3: note = n is u
  source 1..30: mol_type = other DNA

SEQ ID NO: 16 - DNA, 30 bp, synthetic construct; identical to SEQ ID NO: 7
  misc_feature 1..30: note = Synthetic oligomer
  misc_feature 3: note = n is u
  source 1..30: mol_type = other DNA

SEQ ID NO: 17 - DNA, 22 bp, synthetic construct
  misc_feature 1..22: note = Synthetic oligomer
  source 1..22: mol_type = other DNA
tacaaagcgggatcccaatatt

SEQ ID NO: 18 - DNA, 36 bp, synthetic construct
  misc_feature 1..36: note = Synthetic oligomer
  misc_feature 9: note = n is u
  source 1..36: mol_type = other DNA
agagatctnacacaattaatagagaagtcatgcaac

SEQ ID NO: 19 - DNA, 34 bp, synthetic construct
  misc_feature 1..34: note = Synthetic oligomer
  misc_feature 7: note = n is u
  source 1..34: mol_type = other DNA
agatctnacacaattaatagagaagtcatgcaac

SEQ ID NO: 20 - DNA, 37 bp, synthetic construct
  misc_feature 1..37: note = Synthetic oligomer
  source 1..37: mol_type = other DNA
cagagatctyacacaattaatagagaagtcatgcaac

SEQ ID NO: 21 - DNA, 30 bp, synthetic construct
  misc_feature 1..30: note = Synthetic oligomer
  misc_feature 4..29: note = n is u
  source 1..30: mol_type = other DNA
gaangngnnaannancncnncagnacgnng

SEQ ID NO: 22 - DNA, 19 bp, synthetic construct
  misc_feature 1..19: note = Synthetic oligomer
  source 1..19: mol_type = other DNA
cctacgggacatctccaga

SEQ ID NO: 23 - DNA, 30 bp, synthetic construct
  misc_feature 1..30: note = Synthetic oligomer
  misc_feature 4..29: note = n is u
  source 1..30: mol_type = other DNA
gagngngnnaannancncnncagnacgnng

SEQ ID NO: 24 - DNA, 23 bp, synthetic construct
  misc_feature 1..23: note = Synthetic oligomer
  source 1..23: mol_type = other DNA
gagcatcattgcaaacactctga

SEQ ID NO: 25 - DNA, 20 bp, synthetic construct
  misc_feature 1..20: note = Synthetic oligomer
  source 1..20: mol_type = other DNA
acaagatctacaagttggca

SEQ ID NO: 26 - DNA, 26 bp, synthetic construct
  misc_feature 1..26: note = Synthetic oligomer
  source 1..26: mol_type = other DNA
agcaagttacaattaggaataattga

SEQ ID NO: 27 - DNA, 26 bp, synthetic construct
  misc_feature 1..26: note = Synthetic oligomer
  source 1..26: mol_type = other DNA
agcaagttacaattaggaataattga

SEQ ID NO: 28 - DNA, 23 bp, synthetic construct
  misc_feature 1..23: note = Synthetic oligomer
  misc_feature 15: note = n is u
  source 1..23: mol_type = other DNA
catggcataatgtgntatcaaga

SEQ ID NO: 29 - DNA, 26 bp, synthetic construct
  misc_feature 1..26: note = Synthetic oligomer
  source 1..26: mol_type = other DNA
agcaagttacaattaggaataattga

SEQ ID NO: 30 - DNA, 26 bp, synthetic construct
  misc_feature 1..26: note = Synthetic oligomer
  source 1..26: mol_type = other DNA
agcaagttacaattaggaataattga

SEQ ID NO: 31 - DNA, 27 bp, synthetic construct
  misc_feature 1..27: note = Synthetic oligomer
  source 1..27: mol_type = other DNA
ccaggaaacaaygaatgtccatgggga

SEQ ID NO: 32 - DNA, 27 bp, synthetic construct
  misc_feature 1..27: note = Synthetic oligomer
  misc_feature 12: note = n is u
  source 1..27: mol_type = other DNA
ccaggaaacaangaatgtccatgggga

SEQ ID NO: 33 - DNA, 27 bp, synthetic construct
  misc_feature 1..27: note = Synthetic oligomer
  source 1..27: mol_type = other DNA
ccaggaaacaatgaatgtccatgggga

SEQ ID NO: 34 - DNA, 27 bp, synthetic construct
  misc_feature 1..27: note = Synthetic oligomer
  misc_feature 3..27: note = n is u
  source 1..27: mol_type = other DNA
ggnccnnngnnacnnacaggnaccccn

SEQ ID NO: 35 - DNA, 27 bp, synthetic construct
  misc_feature 1..27: note = Synthetic oligomer
  misc_feature 3..27: note = n is u
  source 1..27: mol_type = other DNA
ggnccnnngnngcnnacaggnaccccn

SEQ ID NO: 36 - DNA, 20 bp, synthetic construct
  misc_feature 1..20: note = Synthetic oligomer
  source 1..20: mol_type = other DNA
cacattatgccatgtccatt

SEQ ID NO: 37 - DNA, 23 bp, synthetic construct
  misc_feature 1..23: note = Synthetic oligomer
  misc_feature 18: note = n is u
  source 1..23: mol_type = other DNA
ggatatgcatcagtatanactcc

SEQ ID NO: 38 - DNA, 27 bp, synthetic construct
  misc_feature 1..27: note = Synthetic oligomer
  source 1..27: mol_type = other DNA
tgtgattggtgttgttgaatccggtag

SEQ ID NO: 39 - DNA, 27 bp, synthetic construct
  misc_feature 1..27: note = Synthetic oligomer
  source 1..27: mol_type = other DNA
tgtgattggtrttgttgaatccggtag

SEQ ID NO: 40 - DNA, 23 bp, synthetic construct
  misc_feature 1..23: note = Synthetic oligomer
  misc_feature 16: note = n is u
  source 1..23: mol_type = other DNA
aaagcaggttgaagangtatatg

SEQ ID NO: 41 - DNA, 27 bp, synthetic construct
  misc_feature 1..27: note = Synthetic oligomer
  misc_feature 1..25: note = n is u
  source 1..27: mol_type = other DNA
ngngannggngnngnngaanccggnag

SEQ ID NO: 42 - DNA, 27 bp, synthetic construct
  misc_feature 1..27: note = Synthetic oligomer
  misc_feature 1..25: note = n is u
  source 1..27: mol_type = other DNA
ngngannggnrnngnngaanccggnag

SEQ ID NO: 43 - DNA, 27 bp, synthetic construct
  misc_feature 1..27: note = Synthetic oligomer
  misc_feature 5..26: note = n is u
  source 1..27: mol_type = other DNA
acacnaaccacaacaacnnaggccanc

SEQ ID NO: 44 - DNA, 23 bp, synthetic construct
  misc_feature 1..23: note = Synthetic oligomer
  misc_feature 19: note = n is u
  source 1..23: mol_type = other DNA
aaatgagtccaaccgaacnaatc

SEQ ID NO: 45 - DNA, 27 bp, synthetic construct
  misc_feature 1..27: note = Synthetic oligomer
  misc_feature 5..26: note = n is u
  source 1..27: mol_type = other DNA
acacnaaccaaaacaacnnaggccanc

SEQ ID NO: 46 - DNA, 26 bp, synthetic construct
  misc_feature 1..26: note = Synthetic oligomer
  source 1..26: mol_type = other DNA
agcataattttgtcaactttyccytc

SEQ ID NO: 47 - DNA, 30 bp, synthetic construct
  misc_feature 1..30: note = Synthetic oligomer
  source 1..30: mol_type = other DNA
cattytttgtttgctgaattrtrttttgag

SEQ ID NO: 48 - DNA, 21 bp, synthetic construct
  misc_feature 1..21: note = Synthetic oligomer
  source 1..21: mol_type = other DNA
ctcaattgtkgmaagtgarcc

SEQ ID NO: 49 - DNA, 28 bp, synthetic construct
  misc_feature 1..28: note = Synthetic oligomer
  source 1..28: mol_type = other DNA
ccattattttcattgtygtrattargcc

SEQ ID NO: 50 - DNA, 23 bp, synthetic construct
  misc_feature 1..23: note = Synthetic oligomer
  source 1..23: mol_type = other DNA
cttactttkgatgggactccrgg

SEQ ID NO: 51 - DNA, 28 bp, synthetic construct
  misc_feature 1..28: note = Synthetic oligomer
  source 1..28: mol_type = other DNA
caagtgtaattgtattgtcttgatcaac

SEQ ID NO: 52 - DNA, 23 bp, synthetic construct
  misc_feature 1..23: note = Synthetic oligomer
  source 1..23: mol_type = other DNA
gttccagayaasatgggtcttgc

SEQ ID NO: 53 - DNA, 23 bp, synthetic construct
  misc_feature 1..23: note = Synthetic oligomer
  source 1..23: mol_type = other DNA
gacytcaagaagrccagtttgag

SEQ ID NO: 54 - DNA, 27 bp, synthetic construct
  misc_feature 1..27: note = Synthetic oligomer
  source 1..27: mol_type = other DNA
cagctatttcyaatgsrtcatcaggag

SEQ ID NO: 55 - DNA, 31 bp, synthetic construct
  misc_feature 1..31: note = Synthetic oligomer
  source 1..31: mol_type = other DNA
cagtgctaaattrtctacataattragyaag

SEQ ID NO: 56 - DNA, 21 bp, synthetic construct
  misc_feature 1..21: note = Synthetic oligomer
  source 1..21: mol_type = other DNA
ctggcatctgtttgcagttga

SEQ ID NO: 57 - DNA, 26 bp, synthetic construct
  misc_feature 1..26: note = Synthetic oligomer
  source 1..26: mol_type = other DNA
ctctcstcaactgagaaaacatcatg

SEQ ID NO: 58 - DNA, 23 bp, synthetic construct
  misc_feature 1..23: note = Synthetic oligomer
  source 1..23: mol_type = other DNA
catagattcrcgsactttcccyg

SEQ ID NO: 59 - DNA, 21 bp, synthetic construct
  misc_feature 1..21: note = Synthetic oligomer
  source 1..21: mol_type = other DNA
ctcaattgtkgmaagtgarcc

SEQ ID NO: 60 - DNA, 29 bp, synthetic construct
  misc_feature 1..29: note = Synthetic oligomer
  source 1..29: mol_type = other DNA
cattctcataatrcataacaaytctgcag

SEQ ID NO: 61 - DNA, 28 bp, synthetic construct
  misc_feature 1..28: note = Synthetic oligomer
  source 1..28: mol_type = other DNA
ccattattttcattgtygtrattargcc

SEQ ID NO: 62 - DNA, 23 bp, synthetic construct
  misc_feature 1..23: note = Synthetic oligomer
  source 1..23: mol_type = other DNA
catagattcrcgsactttcccyg

SEQ ID NO: 63 - DNA, 24 bp, synthetic construct
  misc_feature 1..24: note = Synthetic oligomer
  source 1..24: mol_type = other DNA
cttgacaygatctcatytgcttyg

SEQ ID NO: 64 - DNA, 26 bp, synthetic construct
  misc_feature 1..26: note = Synthetic oligomer
  source 1..26: mol_type = other DNA
ccrttytctctraataatttycctgc

SEQ ID NO: 65 - DNA, 26 bp, synthetic construct
  misc_feature 1..26: note = Synthetic oligomer
  source 1..26: mol_type = other DNA
catgatgttttctcagttgawgagag

SEQ ID NO: 66 - DNA, 21 bp, synthetic construct
  misc_feature 1..21: note = Synthetic oligomer
  source 1..21: mol_type = other DNA
cargaaagaggcytgggttac

SEQ ID NO: 67 - DNA, 29 bp, synthetic construct
  misc_feature 1..29: note = Synthetic oligomer
  source 1..29: mol_type = other DNA
ctgcagarttgttatgyattatgagaatg

SEQ ID NO: 68 - DNA, 27 bp, synthetic construct
  misc_feature 1..27: note = Synthetic oligomer
  source 1..27: mol_type = other DNA
gaagtrgcaytraaatactggaaatgg

SEQ ID NO: 69 - DNA, 26 bp, synthetic construct
  misc_feature 1..26: note = Synthetic oligomer
  source 1..26: mol_type = other DNA
garggraaagttgacaaaattatgct

SEQ ID NO: 70 - DNA, 30 bp, synthetic construct
  misc_feature 1..30: note = Synthetic oligomer
  source 1..30: mol_type = other DNA
ctcaaaayayaattcagcaaacaaaraatg

SEQ ID NO: 71 - DNA, 28 bp, synthetic construct
  misc_feature 1..28: note = Synthetic oligomer
  source 1..28: mol_type = other DNA
atcaacccactggatctgaagagagaag

SEQ ID NO: 72 - DNA, 21 bp, synthetic construct
  misc_feature 1..21: note = Synthetic oligomer
  source 1..21: mol_type = other DNA
ggytcacttkcmacaattgag

SEQ ID NO: 73 - DNA, 28 bp, synthetic construct
  misc_feature 1..28: note = Synthetic oligomer
  source 1..28: mol_type = other DNA
ggcytaatyacracaatgaaaataatgg

SEQ ID NO: 74 - DNA, 22 bp, synthetic construct
  misc_feature 1..22: note = Synthetic oligomer
  source 1..22: mol_type = other DNA
aaagaattaggtgcaaccartc

SEQ ID NO: 75 - DNA, 21 bp, synthetic construct
  misc_feature 1..21: note = Synthetic oligomer
  source 1..21: mol_type = other DNA
gctgcttatgggaycagacac

SEQ ID NO: 76 - DNA, 23 bp, synthetic construct
  misc_feature 1..23: note = Synthetic oligomer
  source 1..23: mol_type = other DNA
crgggaaagtwcgygaatctatg

SEQ ID NO: 77 - DNA, 24 bp, synthetic construct
  misc_feature 1..24: note = Synthetic oligomer
  source 1..24: mol_type = other DNA
gtccrtcaaagacytatcaaggac

SEQ ID NO: 78 - DNA, 24 bp, synthetic construct
  misc_feature 1..24: note = Synthetic oligomer
  source 1..24: mol_type = other DNA
aatacaggtttggataatggtgtg

SEQ ID NO: 79 - DNA, 23 bp, synthetic construct
  misc_feature 1..23: note = Synthetic oligomer
  source 1..23: mol_type = other DNA
cctgaagatcttggaccyytatc

SEQ ID NO: 80 - DNA, 23 bp, synthetic construct
  misc_feature 1..23: note = Synthetic oligomer
  source 1..23: mol_type = other DNA
ccctcattgagrgagrtagaycc

SEQ ID NO: 81 - DNA, 21 bp, synthetic construct
  misc_feature 1..21: note = Synthetic oligomer
  source 1..21: mol_type = other DNA
gtattggccacgacctcttca

SEQ ID NO: 82 - DNA, 21 bp, synthetic construct
  misc_feature 1..21: note = Synthetic oligomer
  source 1..21: mol_type = other DNA
tattggccacgacctcttcag

SEQ ID NO: 83 - DNA, 29 bp, synthetic construct
  misc_feature 1..29: note = Synthetic oligomer
  source 1..29: mol_type = other DNA
caaggaaagayttatttacwagtgctagg

SEQ ID NO: 84 - DNA, 27 bp, synthetic construct
  misc_feature 1..27: note = Synthetic oligomer
  source 1..27: mol_type = other DNA
gaatcrarctggaayaagaatcattgg

SEQ ID NO: 85 - DNA, 23 bp, synthetic construct
  misc_feature 1..23: note = Synthetic oligomer
  source 1..23: mol_type = other DNA
ctcaaactggycttcttgargtc

SEQ ID NO: 86 - DNA, 31 bp, synthetic construct
  misc_feature 1..31: note = Synthetic oligomer
  source 1..31: mol_type = other DNA
cttrctyaattatgtagayaatttagcactg

SEQ ID NO: 87 - DNA, 21 bp, synthetic construct
  misc_feature 1..21: note = Synthetic oligomer
  source 1..21: mol_type = other DNA
ggytcacttkcmacaattgag

SEQ ID NO: 88 - DNA, 24 bp, synthetic construct
  misc_feature 1..24: note = Synthetic oligomer
  source 1..24: mol_type = other DNA
ccrtcaaagacytatcaaggactc

SEQ ID NO: 89 - DNA, 27 bp, synthetic construct
  misc_feature 1..27: note = Synthetic oligomer
  source 1..27: mol_type = other DNA
caaggactcattcttgatgcaaaraag

SEQ ID NO: 90 - DNA, 26 bp, synthetic construct
  misc_feature 1..26: note = Synthetic oligomer
  source 1..26: mol_type = other DNA
agcataattttgtcaactttyccytc

SEQ ID NO: 91 - DNA, 30 bp, synthetic construct; identical to SEQ ID NO: 47
  misc_feature 1..30: note = Synthetic oligomer
  source 1..30: mol_type = other DNA

SEQ ID NO: 92 - DNA, 26 bp, synthetic construct
  misc_feature 1..26: note = Synthetic oligomer
  source 1..26: mol_type = other DNA
ctctcstcaactgagaaaacatcatg

SEQ ID NO: 93 - DNA, 23 bp, synthetic construct
  misc_feature 1..23: note = Synthetic oligomer
  source 1..23: mol_type = other DNA
cttactttkgatgggactccrgg

SEQ ID NO: 94 - DNA, 27 bp, synthetic construct
  misc_feature 1..27: note = Synthetic oligomer
  source 1..27: mol_type = other DNA
ccatttccagtatttyartgcyacttc

SEQ ID NO: 95 - DNA, 28 bp, synthetic construct
  misc_feature 1..28: note = Synthetic oligomer
  source 1..28: mol_type = other DNA
caagtgtaattgtattgtcttgatcaac

SEQ ID NO: 96 - DNA, 23 bp, synthetic construct
  misc_feature 1..23: note = Synthetic oligomer
  source 1..23: mol_type = other DNA
gttccagayaasatgggtcttgc

SEQ ID NO: 97 - DNA, 23 bp, synthetic construct
  misc_feature 1..23: note = Synthetic oligomer
  source 1..23: mol_type = other DNA
cctgaagatcttggaccyytatc

SEQ ID NO: 98 - DNA, 23 bp, synthetic construct
  misc_feature 1..23: note = Synthetic oligomer
  source 1..23: mol_type = other DNA
ccctcattgagrgagrtagaycc

SEQ ID NO: 99 - DNA, 21 bp, synthetic construct
  misc_feature 1..21: note = Synthetic oligomer
  source 1..21: mol_type = other DNA
gtattggccacgacctcttca

SEQ ID NO: 100 - DNA, 21 bp, synthetic construct
  misc_feature 1..21: note = Synthetic oligomer
  source 1..21: mol_type = other DNA
tattggccacgacctcttcag

SEQ ID NO: 101 - DNA, 29 bp, synthetic construct
  misc_feature 1..29: note = Synthetic oligomer
  source 1..29: mol_type = other DNA
caaggaaagayttatttacwagtgctagg

SEQ ID NO: 102 - DNA, 27 bp, synthetic construct
  misc_feature 1..27: note = Synthetic oligomer
  source 1..27: mol_type = other DNA
gaatcrarctggaayaagaatcattgg

SEQ ID NO: 103 - DNA, 23 bp, synthetic construct
  misc_feature 1..23: note = Synthetic oligomer
  source 1..23: mol_type = other DNA
ctcaaactggycttcttgargtc

SEQ ID NO: 104 - DNA, 31 bp, synthetic construct; identical to SEQ ID NO: 86
  misc_feature 1..31: note = Synthetic oligomer
  source 1..31: mol_type = other DNA

SEQ ID NO: 105 - DNA, 26 bp, synthetic construct
  misc_feature 1..26: note = Synthetic oligomer
  source 1..26: mol_type = other DNA
catgatgttttctcagttgawgagag

SEQ ID NO: 106 - DNA, 29 bp, synthetic construct
  misc_feature 1..29: note = Synthetic oligomer
  source 1..29: mol_type = other DNA
ctgcagarttgttatgyattatgagaatg

SEQ ID NO: 107 - DNA, 23 bp, synthetic construct
  misc_feature 1..23: note = Synthetic oligomer
  source 1..23: mol_type = other DNA
crgggaaagtwcgygaatctatg

SEQ ID NO: 108 - DNA, 27 bp, synthetic construct
  misc_feature 1..27: note = Synthetic oligomer
  source 1..27: mol_type = other DNA
gaagtrgcaytraaatactggaaatgg

SEQ ID NO: 109 - DNA, 23 bp, synthetic construct
  misc_feature 1..23: note = Synthetic oligomer
  source 1..23: mol_type = other DNA
gacytcaagaagrccagtttgag

SEQ ID NO: 110 - DNA, 31 bp, synthetic construct; identical to SEQ ID NO: 55
  misc_feature 1..31: note = Synthetic oligomer
  source 1..31: mol_type = other DNA

SEQ ID NO: 111 - DNA, 29 bp, synthetic construct
  misc_feature 1..29: note = Synthetic oligomer
  source 1..29: mol_type = other DNA
cattctcataatrcataacaaytctgcag

SEQ ID NO: 112 - DNA, 27 bp, synthetic construct
  misc_feature 1..27: note = Synthetic oligomer
  source 1..27: mol_type = other DNA
ccatttccagtatttyartgcyacttc

SEQ ID NO: 113 - DNA, 24 bp, synthetic construct
  misc_feature 1..24: note = Synthetic oligomer
  source 1..24: mol_type = other DNA
cttgacaygatctcatytgcttyg

SEQ ID NO: 114 - DNA, 26 bp, synthetic construct
  misc_feature 1..26: note = Synthetic oligomer
  source 1..26: mol_type = other DNA
ccrttytctctraataatttycctgc

SEQ ID NO: 115 - DNA, 27 bp, synthetic construct
  misc_feature 1..27: note = Synthetic oligomer
  source 1..27: mol_type = other DNA
cagctatttcyaatgsrtcatcaggag

SEQ ID NO: 116 - DNA, 26 bp, synthetic construct
  misc_feature 1..26: note = Synthetic oligomer
  source 1..26: mol_type = other DNA
garggraaagttgacaaaattatgct

SEQ ID NO: 117 - DNA, 30 bp, synthetic construct; identical to SEQ ID NO: 70
  misc_feature 1..30: note = Synthetic oligomer
  source 1..30: mol_type = other DNA

SEQ ID NO: 118 - DNA, 28 bp, synthetic construct
  misc_feature 1..28: note = Synthetic oligomer
  source 1..28: mol_type = other DNA
ggcytaatyacracaatgaaaataatgg

SEQ ID NO: 119 - DNA, 22 bp, synthetic construct
  misc_feature 1..22: note = Synthetic oligomer
  source 1..22: mol_type = other DNA
aaagaattaggtgcaaccartc

SEQ ID NO: 120 - DNA, 21 bp, synthetic construct
  misc_feature 1..21: note = Synthetic oligomer
  source 1..21: mol_type = other DNA
gctgcttatgggaycagacac

SEQ ID NO: 121 - DNA, 24 bp, synthetic construct
  misc_feature 1..24: note = Synthetic oligomer
  source 1..24: mol_type = other DNA
gtccrtcaaagacytatcaaggac

SEQ ID NO: 122 - DNA, 24 bp, synthetic construct
  misc_feature 1..24: note = Synthetic oligomer
  source 1..24: mol_type = other DNA
ccrtcaaagacytatcaaggactc

SEQ ID NO: 123 - DNA, 27 bp, synthetic construct
  misc_feature 1..27: note = Synthetic oligomer
  source 1..27: mol_type = other DNA
caaggactcattcttgatgcaaaraag

SEQ ID NO: 124 - DNA, 21 bp, synthetic construct
  misc_feature 1..21: note = Synthetic oligomer
  source 1..21: mol_type = other DNA
cargaaagaggcytgggttac

SEQ ID NO: 125 - DNA, 37 bp, synthetic construct
  misc_feature 1..37: note = Synthetic oligomer
  misc_feature 10: note = n is u
  source 1..37: mol_type = other DNA
cagagatctnacacaattaatagagaagtcatgcaac